European Patent Specification EP 3 728 563 B1, published June 18, 2025. Title: FUNCTIONALLY ENHANCED DERIVATIVE CELLS AND USE THEREOF. Applicant: FATE THERAPEUTICS, INC. Application TBA. The sequence listing filed with the application follows.

SEQUENCE LISTING (21 sequences)

SEQ ID NO: 1 - DNA, 19 bp, Homo sapiens
  targeting sequence for CD38 Exon 1 knockout (CD38-gNA-1A)
ttgacgcatcgcgccagga

SEQ ID NO: 2 - DNA, 19 bp, Homo sapiens
  targeting sequence for CD38 Exon 1 knockout (CD38-gNA-1B)
attcatcctgagatgaggt

SEQ ID NO: 3 - DNA, 19 bp, Homo sapiens
  targeting sequence for CD38 Exon 1 knockout (CD38-gNA-2A)
actgacgccaagacagagt

SEQ ID NO: 4 - DNA, 19 bp, Homo sapiens
  targeting sequence for CD38 Exon 1 knockout (CD38-gNA-2B)
ctggtcctgatcctcgtcg

SEQ ID NO: 5 - DNA, 19 bp, Homo sapiens
  targeting sequence for CD38 Exon 1 knockout (CD38-gNA-3A)
tcctagagagccggcagca

SEQ ID NO: 6 - DNA, 19 bp, Homo sapiens
  targeting sequence for CD38 Exon 1 knockout (CD38-gNA-3B)
ggagagcccaactctgtct

SEQ ID NO: 7 - protein, 340 aa, Artificial Sequence
  340 a.a. CD64 domain-based construction
MWFLTTLLLWVPVDGQVDTTKAVITLQPPWVSVFQEETVTLHCEVLHLPGSSSTQWFLNGTATQTSTPSYRITSASVNDSGEYRCQRGLSGRSDPIQLEIHRGWLLLQVSSRVFTEGEPLALRCHAWKDKLVYNVLYYRNGKAFKFFHWNSNLTILKTNISHNGTYHCSGMGKHRYTSAGISVTVKELFPAPVLNASVTSPLLEGNLVTLSCETKLLLQRPGLQLYFSFYMGSKTLRGRNTSSEYQILTARREDSGLYWCEAATEDGNVLKRSPELELQVLGLQLPTPVWFHYQVSFCLVMVLLFAVDTGLYFSVKTNIRSSTRDWKDHKFKWRKDPQDK

SEQ ID NO: 8 - protein, 336 aa, Artificial Sequence
  336 a.a. CD64 exon-based construction
MWFLTTLLLWVPVDGQVDTTKAVITLQPPWVSVFQEETVTLHCEVLHLPGSSSTQWFLNGTATQTSTPSYRITSASVNDSGEYRCQRGLSGRSDPIQLEIHRGWLLLQVSSRVFTEGEPLALRCHAWKDKLVYNVLYYRNGKAFKFFHWNSNLTILKTNISHNGTYHCSGMGKHRYTSAGISVTVKELFPAPVLNASVTSPLLEGNLVTLSCETKLLLQRPGLQLYFSFYMGSKTLRGRNTSSEYQILTARREDSGLYWCEAATEDGNVLKRSPELELQVLGLFFPPGYQVSFCLVMVLLFAVDTGLYFSVKTNIRSSTRDWKDHKFKWRKDPQDK

SEQ ID NO: 9 - protein, 335 aa, Artificial Sequence
  335 a.a. CD64 exon-based construction
MWFLTTLLLWVPVDGQVDTTKAVITLQPPWVSVFQEETVTLHCEVLHLPGSSSTQWFLNGTATQTSTPSYRITSASVNDSGEYRCQRGLSGRSDPIQLEIHRGWLLLQVSSRVFTEGEPLALRCHAWKDKLVYNVLYYRNGKAFKFFHWNSNLTILKTNISHNGTYHCSGMGKHRYTSAGISVTVKELFPAPVLNASVTSPLLEGNLVTLSCETKLLLQRPGLQLYFSFYMGSKTLRGRNTSSEYQILTARREDSGLYWCEAATEDGNVLKRSPELELQVLGFFPPGYQVSFCLVMVLLFAVDTGLYFSVKTNIRSSTRDWKDHKFKWRKDPQDK

SEQ ID NO: 10 - DNA, 1032 bp, Artificial Sequence
  exemplifying sequence encoding 340 a.a. CD64 domain-based construction
cttggagacaacatgtggttcttgacaactctgctcctttgggttccagttgatgggcaagtggacaccacaaaggcagtgatcactttgcagcctccatgggtcagcgtgttccaagaggaaaccgtaaccttgcattgtgaggtgctccatctgcctgggagcagctctacacagtggtttctcaatggcacagccactcagacctcgacccccagctacagaatcacctctgccagtgtcaatgacagtggtgaatacaggtgccagagaggtctctcagggcgaagtgaccccatacagctggaaatccacagaggctggctactactgcaggtctccagcagagtcttcacggaaggagaacctctggccttgaggtgtcatgcgtggaaggataagctggtgtacaatgtgctttactatcgaaatggcaaagcctttaagtttttccactggaattctaacctcaccattctgaaaaccaacataagtcacaatggcacctaccattgctcaggcatgggaaagcatcgctacacatcagcaggaatatctgtcactgtgaaagagctatttccagctccagtgctgaatgcatctgtgacatccccactcctggaggggaatctggtcaccctgagctgtgaaacaaagttgctcttgcagaggcctggtttgcagctttacttctccttctacatgggcagcaagaccctgcgaggcaggaacacatcctctgaataccaaatactaactgctagaagagaagactctgggttatactggtgcgaggctgccacagaggatggaaatgtccttaagcgcagccctgagttggagcttcaagtgcttggcctccagttaccaactcctgtctggtttcattaccaagtctctttctgcttggtgatggtactcctttttgcagtggacacaggactatatttctctgtgaagacaaacattcgaagctcaacaagagactggaaggaccataaatttaaatggagaaaggaccctcaagacaaa

SEQ ID NO: 11 - DNA, 1020 bp, ARTIFICIAL SEQUENCE
  exemplifying sequence encoding 336 a.a. CD64 exon-based construction
cttggagacaacatgtggttcttgacaactctgctcctttgggttccagttgatgggcaagtggacaccacaaaggcagtgatcactttgcagcctccatgggtcagcgtgttccaagaggaaaccgtaaccttgcattgtgaggtgctccatctgcctgggagcagctctacacagtggtttctcaatggcacagccactcagacctcgacccccagctacagaatcacctctgccagtgtcaatgacagtggtgaatacaggtgccagagaggtctctcagggcgaagtgaccccatacagctggaaatccacagaggctggctactactgcaggtctccagcagagtcttcacggaaggagaacctctggccttgaggtgtcatgcgtggaaggataagctggtgtacaatgtgctttactatcgaaatggcaaagcctttaagtttttccactggaattctaacctcaccattctgaaaaccaacataagtcacaatggcacctaccattgctcaggcatgggaaagcatcgctacacatcagcaggaatatctgtcactgtgaaagagctatttccagctccagtgctgaatgcatctgtgacatccccactcctggaggggaatctggtcaccctgagctgtgaaacaaagttgctcttgcagaggcctggtttgcagctttacttctccttctacatgggcagcaagaccctgcgaggcaggaacacatcctctgaataccaaatactaactgctagaagagaagactctgggttatactggtgcgaggctgccacagaggatggaaatgtccttaagcgcagccctgagttggagcttcaagtgcttggtttgttctttccacctgggtaccaagtctctttctgcttggtgatggtactcctttttgcagtggacacaggactatatttctctgtgaagacaaacattcgaagctcaacaagagactggaaggaccataaatttaaatggagaaaggaccctcaagacaaa

SEQ ID NO: 12 - DNA, 1005 bp, ARTIFICIAL SEQUENCE
  exemplifying sequence encoding 335 a.a. CD64 exon-based construction
atgtggttcttgacaactctgctcctttgggttccagttgatgggcaagtggacaccacaaaggcagtgatcactttgcagcctccatgggtcagcgtgttccaagaggaaaccgtaaccttgcactgtgaggtgctccatctgcctgggagcagctctacacagtggtttctcaatggcacagccactcagacctcgacccccagctacagaatcacctctgccagtgtcaatgacagtggtgaatacaggtgccagagaggtctctcagggcgaagtgaccccatacagctggaaatccacagaggctggctactactgcaggtctccagcagagtcttcacggaaggagaacctctggccttgaggtgtcatgcgtggaaggataagctggtgtacaatgtgctttactatcgaaatggcaaagcctttaagtttttccactggaactctaacctcaccattctgaaaaccaacataagtcacaatggcacctaccattgctcaggcatgggaaagcatcgctacacatcagcaggaatatctgtcactgtgaaagagctatttccagctccagtgctgaatgcatctgtgacatccccactcctggaggggaatctggtcaccctgagctgtgaaacaaagttgctcttgcagaggcctggtttgcagctttacttctccttctacatgggcagcaagaccctgcgaggcaggaacacatcctctgaataccaaatactaactgctagaagagaagactctgggttatactggtgcgaggctgccacagaggatggaaatgtccttaagcgcagccctgagttggagcttcaagtgcttggcttctttccacctgggtaccaagtctctttctgcttggtgatggtactcctttttgcagtggacacaggactatatttctctgtgaagacaaacattcgaagctcaacaagagactggaaggaccataaatttaaatggagaaaggaccctcaagacaaa

SEQ ID NO: 13 - protein, 153 aa, Artificial Sequence
  153 a.a. CD28 co-stim + CD3-zeta-ITAM
RSKRSRLLHSDYMNMTPRRPGPTRKHYQPYAPPRDFAAYRSRVKFSRSADAPAYQQGQNQLYNELNLGRREEYDVLDKRRGRDPEMGGKPRRKNPQEGLFNELQKDKMAEAFSEIGMKGERRRGKGHDGLFQGLSTATKDTFDALHMQALPPR

SEQ ID NO: 14 - protein, 219 aa, Artificial Sequence
  219 a.a. CD28 hinge + CD28 TM + CD28 co-stim + CD3-zeta-ITAM
IEVMYPPPYLDNEKSNGTIIHVKGKHLCPSPLFPGPSKPFWVLVVVGGVLACYSLLVTVAFIIFWVRSKRSRLLHSDYMNMTPRRPGPTRKHYQPYAPPRDFAAYRSRVKFSRSADAPAYQQGQNQLYNELNLGRREEYDVLDKRRGRDPEMGGKPRRKNPQEGLFNELQKDKMAEAFSEIGMKGERRRGKGHDGLFQGLSTATKDTFDALHMQALPPR

SEQ ID NO: 15 - protein, 263 aa, Artificial Sequence
  263 a.a NKG2D TM + 2B4 + CD3-zeta
SNLFVASWIAVMIIFRIGMAVAIFCCFFFPSWRRKRKEKQSETSPKEFLTIYEDVKDLKTRRNHEQEQTFPGGGSTIYSMIQSQSSAPTSQEPAYTLYSLIQPSRKSGSRKRNHSPSFNSTIYEVIGKSQPKAQNPARLSRKELENFDVYSRVKFSRSADAPAYKQGQNQLYNELNLGRREEYDVLDKRRGRDPEMGGKPRRKNPQEGLYNELQKDKMAEAYSEIGMKGERRRGKGHDGLYQGLSTATKDTYDALHMQALPPR

SEQ ID NO: 16 - protein, 308 aa, Artificial Sequence
  308 a.a CD8 hinge + NKG2D TM + 2B4 + CD3-zeta
TTTPAPRPPTPAPTIASQPLSLRPEACRPAAGGAVHTRGLDFACDSNLFVASWIAVMIIFRIGMAVAIFCCFFFPSWRRKRKEKQSETSPKEFLTIYEDVKDLKTRRNHEQEQTFPGGGSTIYSMIQSQSSAPTSQEPAYTLYSLIQPSRKSGSRKRNHSPSFNSTIYEVIGKSQPKAQNPARLSRKELENFDVYSRVKFSRSADAPAYKQGQNQLYNELNLGRREEYDVLDKRRGRDPEMGGKPRRKNPQEGLYNELQKDKMAEAYSEIGMKGERRRGKGHDGLYQGLSTATKDTYDALHMQALPPR

SEQ ID NO: 17 - protein, 379 aa, Artificial Sequence
  construct mimicking trans-presentation of IL15 (design 3)
MDWTWILFLVAAATRVHSGIHVFILGCFSAGLPKTEANWVNVISDLKKIEDLIQSMHIDATLYTESDVHPSCKVTAMKCFLLELQVISLESGDASIHDTVENLIILANNSLSSNGNVTESGCKECEELEEKNIKEFLQSFVHIVQMFINTSSGGGSGGGGSGGGGSGGGGSGGGSLQITCPPPMSVEHADIWVKSYSLYSRERYICNSGFKRKAGTSSLTECVLNKATNVAHWTTPSLKCIRDPALVHQRPAPPSTVTTAGVTPQPESLSPSGKEPAASSPSSNNTAATTAAIVPGSQLMPSKSPSTGTTEISSHESSHGTPSQTTAKNWELTASASHQPPGVYPQGHSDTTVAISTSTVLLCGLSAVSLLACYLKSRQ

SEQ ID NO: 18 - DNA, 1140 bp, Artificial Sequence
  an exemplary nucleic acid sequence encoding construct mimicking trans-presentation of IL15 (design 3)
atggactggacctggattctgttcctggtcgcggctgcaacgcgagtccatagcggtatccatgtttttattcttgggtgtttttctgctgggctgcctaagaccgaggccaactgggtaaatgtcatcagtgacctcaagaaaatagaagaccttatacaaagcatgcacattgatgctactctctacactgagtcagatgtacatccctcatgcaaagtgacggccatgaaatgtttcctcctcgaacttcaagtcatatctctggaaagtggcgacgcgtccatccacgacacggtcgaaaacctgataatactcgctaataatagtctctcttcaaatggtaacgtaaccgagtcaggttgcaaagagtgcgaagagttggaagaaaaaaacataaaggagttcctgcaaagtttcgtgcacattgtgcagatgttcattaatacctctagcggcggaggatcaggtggcggtggaagcggaggtggaggctccggtggaggaggtagtggcggaggttctcttcaaataacttgtcctccaccgatgtccgtagaacatgcggatatttgggtaaaatcctatagcttgtacagccgagagcggtatatctgcaacagcggcttcaagcggaaggccggcacaagcagcctgaccgagtgcgtgctgaacaaggccaccaacgtggcccactggaccacccctagcctgaagtgcatcagagatcccgccctggtgcatcagcggcctgcccctccaagcacagtgacaacagctggcgtgaccccccagcctgagagcctgagcccttctggaaaagagcctgccgccagcagccccagcagcaacaatactgccgccaccacagccgccatcgtgcctggatctcagctgatgcccagcaagagccctagcaccggcaccaccgagatcagcagccacgagtctagccacggcaccccatctcagaccaccgccaagaactgggagctgacagccagcgcctctcaccagcctccaggcgtgtaccctcagggccacagcgataccacagtggccatcagcacctccaccgtgctgctgtgtggactgagcgccgtgtcactgctggcctgctacctgaagtccagacagtga

SEQ ID NO: 19 - protein, 242 aa, Artificial Sequence
  fused IL15/mb-Sushi construct (design 4)
MDWTWILFLVAAATRVHSGIHVFILGCFSAGLPKTEANWVNVISDLKKIEDLIQSMHIDATLYTESDVHPSCKVTAMKCFLLELQVISLESGDASIHDTVENLIILANNSLSSNGNVTESGCKECEELEEKNIKEFLQSFVHIVQMFINTSSGGGSGGGGSGGGGSGGGGSGGGSLQITCPPPMSVEHADIWVKSYSLYSRERYICNSGFKRKAGTSSLTECVLNKATNVAHWTTPSLKCIR

SEQ ID NO: 20 - DNA, 726 bp, Artificial Sequence
  an exemplary nucleic acid sequence encoding fused IL15/mb-Sushi construct (design 4)
atggactggacctggattctgttcctggtcgcggctgcaacgcgagtccatagcggtatccatgtttttattcttgggtgtttttctgctgggctgcctaagaccgaggccaactgggtaaatgtcatcagtgacctcaagaaaatagaagaccttatacaaagcatgcacattgatgctactctctacactgagtcagatgtacatccctcatgcaaagtgacggccatgaaatgtttcctcctcgaacttcaagtcatatctctggaaagtggcgacgcgtccatccacgacacggtcgaaaacctgataatactcgctaataatagtctctcttcaaatggtaacgtaaccgagtcaggttgcaaagagtgcgaagagttggaagaaaaaaacataaaggagttcctgcaaagtttcgtgcacattgtgcagatgttcattaatacctctagcggcggaggatcaggtggcggtggaagcggaggtggaggctccggtggaggaggtagtggcggaggttctcttcaaataacttgtcctccaccgatgtccgtagaacatgcggatatttgggtaaaatcctatagcttgtacagccgagagcggtatatctgcaacagcggcttcaagcggaaggccggcacaagcagcctgaccgagtgcgtgctgaacaaggccaccaacgtggcccactggaccacccctagcctgaagtgcatcaga

SEQ ID NO: 21 - protein, 375 aa, Artificial Sequence
  protein construct further modified from SEQ ID NO. 17
MDWTWILFLVAAATRVHSGIHVFILGCFSAGLPKTEANWVNVISDLKKIEDLIQSMHIDATLYTESDVHPSCKVTAMKCFLLELQVISLESGDASIHDTVENLIILANNSLSSNGNVTESGCKECEELEEKNIKEFLQSFVHIVQMFINTSSGGGSGGGGSGGGGSGGGGSGGGSLQITCPPPMSVEHADIWVKSYSLYSRERYICNSGFKRKAGTSSLTECVLNKATNVAHWTTPSLKCIRDPALVHQRPAPPSTVTTAGVTPQPESLSPSGKEPAASSPSSNNTAATTAAIVPGSQLMPSKSPSTGTTEISSHESSHGTPSQTTAKNWELTASASHQPPGVYPQGHSDTTVAISTSTVLLCGLSAVSLLACYL